European Patent Application EP 4 299 726 A1, published January 3, 2024. Title: Novel bacteriophage having a specific bactericidal activity against Clostridium perfringens and antibacterial composition comprising the same. Applicant: CJ CheilJedang Corporation. The sequence listing filed with the application follows.

SEQUENCE LISTING (1 sequence)

SEQ ID NO: 1 - DNA, 51650 bp, bacteriophage CJ_CP_20-15
cttggtcagttggtgggtaatcaaagtatttatataactcaagatcagtaaaaaatctttctagaccttccttaggagtggtcttgggatccacatagtcttgtaattcctgtcccttagtatataacttctgaagttcagtagccataatggtgtttactaagttatcagcctcttttatattatcataaaattcaggaacatacaatagtaattctttttgaacctgttctagactatacataagttaccaccacctcagtaatggttggtatttgattagcaggaatagttaaagattgactacttccattaagtgtaatggttgtataatcttctactccctcaatatttaaaagcatagcccctattctatttatagataggctagtaattttaaatacttgactatttagaaattcttctagttctttcttgaagtttaattttatttgttcttctgtaactgaactcaatttcttaacttgagctcttacagtgatattaaaggtttgggctgactcaacagtaaaaacacatcctataggagctttaccctcacctaaacctttcttgcctggatccatgtattcttgaactttattaactagctcaggattagcaggcttattttcaactgtggttataatacctttagcagtatttattccatcccaacagggaagaaccacagctttacccactccagctacacttttacaccaatcagttaactgttgaacattcccatctccagatggttgtatagtggctttagtagctctttctcttaactcatcatctgtctcctgatctctaccaataacaagtatatctcccatagtagcacttctaagttctgctatagcattgataggaattaaatgtgtacctgttgatactttattgggtcctgaacctaaggtctcacattcaataatattaggctctatcacttgccagaaataatctcctccttggaatcttgaaccaacatcgggttcatagccaacaaatatagctgaccttctacacttagttggaattattctggatatccctacattggcagctctctcatctaagaacttacctgtagcagtacttagaaatactgagtctaatatttgattaacattaacagcataaaactcagctagcttaacagcaaaaaccatagccatatcataggtgaagcttccagttctagtgtcaatatcatcaggggataggcctatcatttcttctaataattctttatgtgttcgggagaataaatcttcagaaaatcccattatatcaccccttccagttttgtatctccatatatggtatttatccatacttcaatatatacattcttaccttgcacattatactttagatcagttactttagtcactctatcatcttctaagagacattcagggatagccctattaatctccatttcaagaagttcaggagttactagagagtcattaatcaaagctctaatatcacaaccataagaagtatcttgataaatcatataggcatttttaggagttattaatcttttatataaagattgttttaaggcctcaagaccatccacattatcataaatcctattaaggtttagatccagtttataggtcttggtattctccattgttttctcatcaactataagagtatctttaaagccattaggtagcattatatcaacctcctaagatccctaacataaaatatctttgtccatcatcatagggcataagataaacagtatcgccctcactaatagactcaatatgttttggaacatctataatatttccagatagtactaattttctattgtgaagacactcacattttagagggctagtactaagtaccttagctctataaatatttagaggggtggacatattactatatacttgttttacacagtctaataaattattagccattaaatatcaccctcctcagtacatttaagttttaaattcatggtgtagtcagtatcaaatttatgggtatcagactcaatgtagaaagccttgttaatttttaaatgtggtatactaaccacaatggctttgccactaatacaatcaggtacacctataacagttatagagatatcagttttaggtctcttacctgtttctagctttattctagccttctcatttaattgggcttggtttagttcatcactgatagtatcgtataattgaaatacaccatatttcttttggctgctatcatctttagcagaggcaaataaagtaatctcgggatcatctttacccttaccctgtttatatttacatactagctttacctggttgacaatactatcaaagtttctacttcttgaaaaggttccaatatttttaccatattcgaatttccacaattcattattggttcttcggtttataaaatcaaacttacctgtaatagaattatagtaaatataaaactgttctccagtttgttcataaacctcttttattaccttcttcataatatcatagggagtttgtttctcacatactaaactagagaaagtatatccagttttagctactactccaggggcaaccccaaaggctttacataatgactcaaatatagcttcgccagtttggttttcgaatacaaagctatctttattattagcccaataaatcatagggtcataagctttaaccttaagtaaatgctttttctcattatctgagatattcataataataccattaaagatattcttaccctcatggactagtactacctgatctccatcataaattggatgtatatcttgagcattatattggaatgatagggtacgaggggcagatgaagaagaccctgcccaactcttaccactggaggtatttgtaatatcaaaggatttatctccttgtaccacaattaattgcatattataacctccttatataatcaccagaactccaaccttctttatatcctgaaccattatctaatttatactttacataatgccatccattttgagatcttaatactgtaaagtgttcattaggccatatcttacccttagtgggattattgatacctggtccagttcttacccatagccatgagtaaacattagtagtagtagctgcccaaggttgagtacctccagaagaactacctcctgtattaccactataggctagtttaggttttggaattgtaaaactaactgatttaacctcaggcttcttatactcagttagttttatttttacttgaagagtaccaatatctccacctttctcagtatatgagatattatcaatagtaactaataagttaatatcagtactagtaatagtaaatcttactggatctttacccatttcaataagtttagcataacttactctagggtctgcaatatcagtatactcacatccatcgtagtatgagcttggtaactcaaaattaaaagaaaaagattttagcttagggtctcctatgaaagagagttcccctaagccttcaatggaaactgtactattatctctactatcagagatatttatatcagtgggatttactggtaacctaaacctagtatctccctgtattaaccagaattgatatttactatgcaaggtccagttcacctccctcgaacatttcctgatttaacatttccacaataaatctgtatactctcattaattcactttctgagattgttccatcttcagcctgtactgtgaaattaaatgagttgttaatgttcataactttagatccatcatcacttcctgctccagattgtcttagtaaatcctgagttttatctgcaggtaatacttgagagcctctaggcatttttgagaatgtaggacccataactaattcaggaccagcttcaccaaccatggcagctttatctgtaaagaagtcagtaccttcagcaagcattggtatctggggaatattaatacccttacccccaataataggtacccagtcaggtatcttaatagtattaagagcaccaattaagttattaatcataccaataatactattaataggagcttttgctagggataacataccttggaaaatacccccaaagatgttcttaacaccttcccaagctttagaccaattacctgtgaatactccagccacaaaagctattaaaccactcaacatctgcattaatccctgtagtattcctgatatagtttgaacggccccagtaacaactgaggagataacaggccatactgtttggaaagatgcggctaaaaggttaagtagtggagttagcatatccaccaacccttggaatatcataccaaaactctcaatagctgattgaatatatggaactacattctcagcaaagcttaagaacataggtagtagtgtattattccaccaatctgctagtccttgtaatattggcattaggaagttacctatagcttccacaacttgtgatatagctggggctatgtaggtgttaaaggcttcagctaatgatacagctattggcatgaaaacattagttatcaattctccaagagctgtaaaagtagcagagaacatagaacctaatacttctaatatagggcctaacacttccaatacagtttgccatacttgagtaaagccttgaacataaagaactactaagtctatggctggaattaggttattcataaatatagaagctaaagttccaaacatatcaagaagtacttgacctataggagctaatactcccatgataggctcagctaaaccattaaaggcttcttgtatattattattagcctctgataaataatctggtagacctattaagatctctccaaaattattatagatgtcttctccaagactccatatcttctcattaatttgatctgccacatcagcaggtaagaacttatataatatatcattggttagatctataaagggttgcatagcatccccaaactcccaaccattcatgatgtaatatatagtctctcctaaaccttggaaagcagaaacaaccattgagaatataggtcctagtttttcaaagccttcttgtataaatgtgataccatttagaacagcattagctataacctcaacggcaggggctagggcatctcccacatctaacataactacagcagctttggtttttattctctccatggttctattaaagcccttatccattttttcataggcagcttcagtggccccagcactatccttcatctcattaagagcattagtaaaggcctcagtaccttcaccagtcaaggctagtgcagctgaaccagcttctacagaaccaaagaggtcattgatacccagattacttttctgggcatgtttttctaacatctgaagggcctcttggatattacctccacctttaatgaagtctttgaagcccttaccagctatttcccggaagactttatcagtcttggttcccgatttagatagctcatctatagcagctcttatcttagtagtagctacagatgttggaaccccctgagctgttaatgcagctatagaggcagatacttcttcaaaagataccccagcagctgaggctgaaggtagcacattgaatagggattgtgatagttgctcaaagttagtcttaccaagtcttactgtagtaaacataaggtctgaggccctttgaacatccatattcttagctccatatgagttaataacagtagttagtccatcaaccgcagtttctattgatgtgataccacctatagaagctttaccagctgtttctaagaaactaaaaacgttatcctctggaactgatgaggatatagcttgataaagagcaggtactactttatcaggcaatatccctatatcagaacttaacttttttacctggccggacatcttatcaaaggtctcttgagtagagttgggtaatagagtcataacctcatttaaaccttgctcaaaatccccaaaggctttaacactgtccttagtaaaatcccagacagccttagctgagaatactccagcagctactccaccaattttggcaagagtacccatgaaggaattaccactatcagccatctggttaaatgcaccagagatcttatcttgggcagagaatatggcagtaaatgccgcttgacttgccattatatccctcctttatgattaagagcctttctttaacttatccctagcttttttatcttcctctaaagccagttcacatgaggctataagaaaggctttcctattgggagatagtttatcaaattcccagggtagtatattatgcttctggaataacacatgagcccaaaatgcactagtgtcggcctttattagttttttgcttctttgattagatcatccttattatcgcctaatccatttatgtccataacctcactagttattctagtgaaatctcctggtaagcttagtacatccataagtaaatctactggatccacaaacttagtagactctaaccattttggatctttaaagtcagggaatactattgtttctagtatcatttccctagtagctcttctttggtctgttattgagttagttatacctttgtttctagtaattactgtatttctcttttggatatcttccatttgcttagtagtgattggctttaatatccaaggtataggttggcccgctaattcatgaccctcagggaaactaaatctagctaccccttcaacttcaatttcgggtgattgtttacccttatcattttccatgaaaaattccatactaaattttgacataataatctacctccacaatattcttaatcttttataaatatcttacttctgaagctgagaatgatatttcttcttgaatttcttctccctcagcatctagtccaattagtggtaaatctccttctaattgtactcctagtaattgtactctgtcctcaccataattcttaacatagtcagaatctggatcatcacatacagcttgtatatccatcttagggaatataccagtttttaagtattccttaatagcttctcttatcattggagtagctttgaattgagttatagttccagttatatcataacctataacttttgaggttaatcctttctgacccataactcttttcttagtcacctcaggagtaaatagagcttctagttttattaagctagttacttgcttacctgatacaaaagctctaccctctctagcagacattctattaacttcactcatgggctatacctccttaattattcttaacagttacaaagtatttcttgaaagttcttacaggttgtgtaagtatagtagcatacatagtctttcctttactagcttcttcatctaccactacatcagagtcagggtccacattctttaatgctccttgagcttgtagtgtagttaatagacttattagtctatcctgagctagctttataccatctttgtggttagggaaaacattaggaactaagatctgagatcctagatctataacagcatccaatacagccacaactttgttatctgtaaagctttcatcccattcttctgtaaaagtatggtgtgtatttatatcttcctcaactactacctttactctttcagaatttgagtcagtttgagttgagaatataaattgacctgtttttaatccatcaactatttgagagtgttttagtcttggattggcatctactgctccaggatatgctttataagtaaggtcttcagtatatccagctgcagctctagcaccagctacccatgcagttgcttgagaagctgttaacttagtgcccccttctaatacaacaccattcttaacattgataatgtatgggtaatcacaagtagcaaagtcagaagtaactgccacaatattcttaccaacttcatctctgaagtatttaagttttgataatagagcagtgtgtaattcactatcagtaaatgggaaggccatagttttaaagttgtataactcacagttatctaagaagttgataacatcagagttattcatctgagtagaagtaccagtactaaactcagtcttagcagtctcatctatagaaccacttccacttactgtaaaccattgagacttaactgttgatatttcagttactcctgtagcctcaaagattttagatccctcaagatataataatatatcctttcctccaagaggattggtcttaatagttagagataacttattacccctttctccagctttagtagctgtaaatgttagagaccctactacagctttggctttagttccacctgttaggttatatactaaaacagttgcagcttcttttaaagcctctttaactagtaatacagtagggtgagttatgtcatacccaagttgatataatgcttctaggccaccttcattggttaccttgataacatctccagcattaccccatttaagttgtaatggtaagatcataactcctagattattaagcttaggctcattaagtccaccacttacgaatctagtatacataccaggtcttactttattttgtcctggaataaaagttcctcctgccatctattttacctccttctttagccagtcttttataatctgactagtttgttttattgttaactcttcatcaggtggaagggattgaactgcagcgttgaagacaaactcctcaacctggaaaagttgttgacaatgggctcttaattgaggtatggaaaatttttgtactttcactattttaccccctttgttatctcaaagttttcgaagtaagttggatctttataaagactaaccacaatatcatagtttatctctacctgagaatcttcttcagtttcaccttcaaatacttccacattctttattttgagatttttgttggtcttactaccatccctattaagtataggaatttttctatttctcaagtatatagcattagctatattctgagcaatttcaagagagtctttaggttcaaataccttaactcttaaagtattctcagttctataactacaaagagtatcattctgaggattaaataccttcttgaaatataatgagggatacttgaacttttcaggtattcgctcaaaatagaggatagtaattccagttagatcagatatgaatttagcaatactccctatatctgctgtcattaataactaccccctaaaacttcggctaaccaatcttctaattttctttggaaagcctgttcaaatattttttcatatatttttactgcattgtcccaataaggtttaccaggtactttcttttgtcttagtaccataccagtcttagctcctggttgataaataaatttatctcctgaccatatgccaggaacgaatctaaatgattgtccttgtggattagtgtagtgaccatcgtttacccacttagcatattttaggttagtaccaacttctaaagttagtcctccatcactacttacccatataccattcttacctcccttttgaaaggagttaagtaataatctagtgtctactacttgtagtctaattatttcatcttgaaccacatcaaggaagtctatccctgcagcttcaaaccatactgctaattgctttttgaaatcactattagctgcatctcttagcttctttataaacctttctatttgtttagcatctatttctatgcctccagaatttgaagccataactatctaaaatccttagcctctataccaaccttaatttttagacctcttatatccctaggagctttagctatatatgtgataccagtctcaaggtccacaattttatcattttgtctaacatcagttccaatagcaaaatctactgagtactcctgggtaatcttaaacctaggttctttgtactcaagtttttctagagttcctgacttaaaatgacagggtacctcagtcatgtctggctcatcaggataactaaagctaggggtatgggctagcccatatccgggatcttcagggtcttctaataggtggtatatattacatctatgatttaagagcttgttatatgaatttccaatcatattacagtacccttaatctcatagtagttgttctgatagatggactatcatcttctaagaaaggtttaatcagaggcataatatcaggctctatgacagccttatcagttcttcttgtatatgagtaatcatcataggtctcggattgaatatcagccttgctaatgaccaaggattgtagtccataatactcagcatacaatatatgggctaaccttaattctttactattaggatttttctccacaatagtatcatagtctttatttgaatttttaaaaattcctgagatcttggctttagctcttagtatatccatctcaatatttttggggtctcttttcttaatctcaggattacttgaaaagtcaattatttcatccggagtaatattcatatgagccacccctatctgtttcttttattcttgtttgtaaatcttctagcaggttcttctttactgtcatctgtagaaggtatttcttctccagtaaaatcttctagaggttcatcctcaacaggttcatctatgacaatcacatcatagttctgttttaaataatttactaggttatctttaacttcttctacatggtcttgagtaattctatgacccttaataaccagagtttgtaatttaccctttgctaatttgaccttagccataatatctctcctttctaatgaaaaagagcccacatttatagtgggccttcatgattaagcttttaccttgattatcttagcagcagctttaggatcttcaaacttaacatccatcttaagagttaaaactacataagtagctctttctctaggagctctttctaattcaattctgatatctcttgatatacctataactatattcttagggtgagttaagattatatctgatacttgagtagaagtatcttcataatcttgtagcatagctatacctttaacaggtacaccataagcagatttaacagagccatttataaatgagtcatcaccattagcagttaatctctctcctactaagtctacccaatcagtttctaaaccatttgagcagtagaatctccactcactggggtttcttaaatacttagctggtacagctttcttagcttgttttaataggtctttacttaaagcacccctttgagcatctactacatgagcagttaactgttttctaaccccatctaattgttgtaagaactcatcactaccctcactagtatcaccattaacaattatttcttccatatcaagagcaactctttcagctaataattgcattacagtgtcttctattgattttccttctatatttgtttctatagtatcatcagttaacttaaccacagctataaattctttagcttgtaaagtaactgttccagtagttggagctgaatatttagactcccctggatcttttccttcagttgcaggatttaatactctttgaccaaatcctattgactcaatctttttagagtctcctttcattggtacagttctagcctcttttaatattgttggctcatcaattatcattttaataaaagcgttagcttgttctgtgtttaatttacctccaccacttaatactgtagagttaaatactgctttatttattttagccataatcttttcctcctatcaattattcttggtttccaccaaataatccattaaatactgatttttgaacttcttgtccttctcctccatttttaacaatttgtttacttcctacatatggagccatggccttagctactgcctcagctattttttcttcctcagttttttcttcttgtttctggattaagccagcctctaacatagctttttccacagccttagcaactatatcttcagtagtagcttgttgaccttcactctttttaacttcaccctcaacaggtttagttccatctaatgcctttttgatagcttcgtctatcattttttgtacttgagtttcattcatctcttcttccccctccactgagtctaataattcattaatagcactttgtgctgtttttaacttttccacattttttgaagatattttcttacctgccttattgactggtaactcaaaggatttagctacttcctcgggagttcctaataatattccctccatagtttcagaaaattcttgaagagcttcctttatcttatctacatcactttcaaaagatctagtgtaatcccaactagaatatggatatagaatatcttctaaggtactaactgcattccagaaattatccctttttgcagtctctttatatttttcagagtatgcacctttctgtatatgctttggagttaaccctaaggcctttccaatcttatcaagtatagattgacctatagacttctcaatctcatcaatatctacatcttgtgtagaatatttaccagtaccacccatagaccatccagtaatttcgcctttctcaatcttgctccatagatcatcatcgacaatctcagctttagctagccaagttccagctttaactactgtaccttctattgtagtatcttcctcagttacccatgattttacaatcttgacaccctcaagagtgttctcattgtgttgtaaatcactaccaaggccattttcattaaaccactcacaagctttcttgatctcttcctcagtcataaaattatcatggtagtcagcagtcattggctcatatactacaccgataacaaaatgattatctccttcagactcagactttaagattggcttatcatatctaaatctattaggagccccaagttctttagccacaatccattgccatttattagctgctttatcaactaatgaaaggtaatcaattttagcatctgagatctcaatagctttcttaactgattttactggcatttactctccctcctttacaaattatattctgctatcacttgatctctgatagcttctttttcttctttagataatcctagtatatccttatcaattacaggcccatgggtacaatgacaattcacagtctcagaagctggtaagttgatatccctaggaaatctagcttcataaattcctacagtgaagtactcacctttattaatgacagtaccatccagatcgacatggtgttgccttgggtgaataccccttccccctgagtgtttccactgtattcctgttactgcggggcattgattaaaagcctcatccttagcatatgaatgagctcttaacatttcagtaatagcagtagctctagctctagttctactaaagccataagtctcagataatttaccaactacatcttctacagactctccatcttcaagagccttatccagaatattctgtagtttttcatgggaagttaatttcatcatttcccctagtttagaagaccactcatctataaaggtagtagtatatggagaaaagactttggttagggataagtccttatcaataccttgtaaataagtatctcctaaattttctatagcttcttgataacaactcttaagagtttctgctaaagaagtatcgatattatctgtacctatttgagactccacatattccataaattcttcaatggtttcaaagtctccatcttttataagatgttttaattcttctgtaaggagatcagaaatagtgtcttctaattcagagatcttttctattgtataatcaatctcctcatagccagcttctttcaattctttcttaaggctatcatcttcattctttaagatcttatcaattttagcgatcaactcatcagtacccactattacttacctccttttaattgatagtttaataactgtttcttagcctctttaagtacagctatcacctcatcactcccattagagctttgagccttctcaattatacttgttaagttattactcattgaagaggcaactgagtaagtagggatatttgcccattcttcatcaataggagtatagtccttattgattgatgaatagtactcctcattaatctgattaggagtcatagctctagaggctatagcaaacattcctttctgataatcagagttctcaatattaggactcttaaagtaagcttccacatatttaaaaccatagccagatagaataacattatttagtatccatgttaggttttctctttcaggaacaaatacttgctcttcagtttttcttgtagcctctctggctgtagccacattataatcttgggagtaccctacatatatatctggtagtaagaaagaagattgtatctttttcctagtattatccatgtagtcttggaataactcatccttctgtaatatttcagataggggcttgacctcaacagtaactggcttagaatcatcaagggcagtgtctctctctgcagcttcagtttctaatactaagaaaccatgctgggaattttcaccttttacattattcatgtactcagttaattcattccaagatttatcattaagagtaccaccttgaattagtaacattaatggagtatgtttaccattagtaaaatatctccagtttaataattcggcctttcttgaaccttgagcggctaacataggaccttcccatcttggtgtaccatagacaccataacctgttttaaaatgaagtatactgttagctcgatctttaagaggtatctctcccttttcataatactttccagtattcatatctagatctctaggatctccccactctttaaagaagattgattgattatttacagtctgcttaaatcttctgaatctttttcttctagtgtactgtttaccatatcgggttacagtgtactctgtactctcatcatctagcttaagaattttaattgtcttagggtcttcaatttcttttatctcttttacgagagctgagtctttaggatcttctacgatctctaaaaaagaatacccaagtccttctctccaatcaactatctcttcaaagacattcttggttggtttatcaaaagacagggtatcaattaattcttccagctgtttatattcagcttccatttctggagtaggttcatctaccttctcaatatacctaatacctattccgaatccagcaatattatttcggtaggcctttttgcattggggtattattgtagactcccttataatcacttctaatagttgggggtcatattcaggggatatctcatcaacttcaattccaagtacactggtttgttgattagatttatccactggatccaaagacttttggatagggtctccacatatacttctggcggatatctttttcaaagttactttacctcctttcttaccttatatatcaaattataaaatccagatggcctcatatttcagggaggattacatcaactccacatatagtgtcaaatacggccattcacatgatttaaaaataactataatttgatacgtttattataacataattcacaaaaatttgtcaacgttttatttttacattattttccagaagattttccgcatatattccccatataaaattatataattattaatgtatactatattactatattaatttatgaaataaattatatagtatatagtatacttatattacatatatataaaggtggtaactctgatatgccttctatatcacattattactaatatagagcctagtcaatttcaaaactgatatctcacatatcagaataaaaattattggctttaataggcatatcagttacttagatttttcttaatttagatccaacaggaaggcaagctaagaatagagagtctgctaagtctggagaatgtagtcctcttttcttcatttcatccttactctccagctttatttgacctttggagttgaatactttaaactttctggtagtcaattctcccacaagatctgtattatctggtagtcttaactcatcatcctccagtaattccttaactacagaggctatatatgtggttgtatcataataaaaggcataagcctgggaccccctctttaatggcataccaaatttacatggtactaccttcaaccagtccagtttttcttcaaattttatctcctttaatctatcagttactcccccacctacaccagtgtcgtctattttcacaactactgctagtttagggaactcaccatgtagggatttagcctttcttagcacttctcctactgttttcatagtgtccttaccttggtaatagataggttcttccacatatccatcaattttggtcataatagaggtcttatctgaaccaaatctagctacgtctacacccatatctatagtaactggttctgtaggtctggttatttcactattaatacctctatatactgtggataattgtataaatatgtcatcttcttctagtgggaagtccccttttaccagacatctgtagacattggactcttctccatactttttccttaacattttatggttttctttatcagttctatcaacttttgtagcgtcaatatgaatacatttaaaattttccttaagactgtggtgagaatcaaagaagatacctgtatttttaacagggttaccaatcaaaattatcttattttcctcatcggatatagtaccaagtaatgcttctagtatctcatcatctattccaggagcctcatcacatataattagcataaactcactatgaagaccaagcatattctcttttctattactagttttacacatagcaaaccaagtcataggactacaattcctagtcatagtagttttatttactgtaaagtaatcttccacaatagttccttgtagccattttgatatttcaggccataatacagatgttaactgtgaaaatgtaggagctgtagcaattaccttacattcaggcctaaaggtcatataccaaattataagacaagcacaggccatggtcttacctaccccctgtcctgaccttacagaggttctcttattgtctcttacactcaataaaatatctttctgatgtggatctaagtgtactcctagtatatcttccgagaatccacaaggatcgtcatagtatagatctactaattcttcaaaggatatttcttccagagcttccttgttaatgtggaacttatcaactaaagcatctagctctaatttctcaattatgctatctaaatcaaacaattatatacacctccttagtaaagtgctttatttagtcctgtaatacctttttacttagtggtattagattttcctttacctgcattctttttctttctatcagccattttggctctaagaacctcaagatcttttcccttaccagcattattctgattttcctgtatttgtaaaagtaatttaaccttttcaagttcaactttcatcacatcagtacttaggccgaagtatacctcaagtctttttagtgcctgaagtctatcctccattttaactgatacgccatctttactttgtttaatctcattgattaaagtaccatctacagccttactagaccttaatagaactagatcatccttgaattggcacacatcagttatatctgcaaaggctattttcatgtactgccttattacatccataccatcgcatagtaattcttcatctctatcggctctgatagcctttagagcttcctgtattttcttcttctttaatagtttagacccatgtgcatgagaattattcccaggataacctgctctagcagctgctgtagttgcattaaagcacttcatgtaatgaaatacaaacaactcttctttctcatcaagatcatacttatcagccagggtcttaatagtcttttttgttttgctactcaatgccacaatatcaccttcttcttctaaaaatgttatgccctgctctttaaactctcttagacactgcctaacaaaggtctgtgataccttagcaaggtttcttagttgtttaggatgtgtaaagggatcagccttcagggcattatatatcaattttttggctttcttcaaatgttcaggagtacagtactctggttcagtgtatgacttatagctcataatacaatatcacccccttaaaatccagactttactacgtgaaaaatggttggcacactaaccttaatgctagtaataccaaccaaatggcaaaattaactatggatttataccactattataccacatctggattaattatgtcaacgttttataattttatttcacctgtcaatattttttcatacatatccacatctattcttccttcctgtagcaggttatcagctgcaatttgtatctcttctggggaatatactggattacctttagtatcaagttctataccagtatatgagtctaccttacctctgttcataccatatccaactgatttatgaacttctagtttttcattatggtcttcttgccagtgttttaattcttcctgatattccttattctcctctttagtttgtttacattcaataggtctattatctttcatcttttgctttagagctgctgtattgggtttacagttcttagatcctccacctgaacctctattcttatcttcctcataagctttattaatctcaatcccaattattagatccatcttctctaccaagtaaagacattcttttactattggattgttaggttgatttttagaaatgatgtcttgacactctttctttaattgatgtggattattacattggctagggcatttttctcctggcccatatggaattgtatatgctaagcagttacctgctggatcccttctataacatcttcttttacatactattttactcatggttaatacctcctaatatattttctttctcttctaataatttttcaagttcctcaagattttcttctttatcactattaccagctttagctatatttagaatagcttctagttgttcctcactcaaaaactcctttaatttctcatcctctaatatattagatacctctttactcatattgttctacctccacatcattacaaattaatttagctattccctcacttaatctgtatttctcaagatataccactttcttaattcctgcattgattattaaattagcacagctctcacatggggataaggttacatacatagtagttccttcagttgagatcccatgtttagcacagtaacttattaagccagcttctgcatggatcacaatatcacatccaggacctaaacaagttttacaatgttctactcctgaaggtactccattatatgaagtagcaactatcctgttatctctaactaatacacaaccaactgcttttcttaggcaagtagatcttcctgtcataagtttagcaacttccatgtaaagtgtttctctgcttattctgttgttattattttccatagtttatcacctcaattttattatatactattccctatcatatgtcaagagaaactttagaaaggtatatcaccataatccagatcaatacattgggctggctttggttttacttttttaggctctggagttttcttgactttatgatactttggagctctggctaaatccttttttaactttctgactctcttcatatcccactcatgtatttcatggtctctaaaatattcattcaatactcttactgcggatctctttgaaggtgtctttacagagcagttattaggagcaagacagcatcctgtctccttatctgatatagtataacatactgtattatgaggggctcctacaggcctatgaatgaataaggttctgcccatataatcaaactcacataatacttccacatatcttttatactgttgtccctggtcattcttacataatacataagtatattctttcatgttaattctcctttctatgttaaaagggagatcatctctccccttaatatctttttattcttctgttgttctcatcaacctcaatcacttcataccttctaaccttatcagatataccttcctcctgtaatactttaggaatatatcctatggcctgtcttttgttatcaacttcaaaatatctggtcaagatcctttttgatgttacaatcactaatcttactttcatattatctacctccatgtggcctgaactacagctccaggtctatgcttagcttcaatcttagcttcttcctcagtatcaaaatagattatatcttccttgtgttcatccttaacagatacccagtgtactcctaaatatttgttatgtgctaatacactaacatcagggttccaatccacatcaactgtaacttgtaaaacgatatatctccttttcatatcagttctcctttttgtatttatttgttgattttattataagagagcctcggaagtttgtcaaagattttctcgaaggaattcgtataatatcttccgagctgagcataatatagactataaaacaaaatcaaggagttgtaataaatgaaagataataatttaataccattaagagatattgccaaagaggttggaataaatgaaaggaaagccagaaagctattaagatcacatgagaataaagcaaatcacaattattattggatgtttacaccaagagagaaaagacatattgtatcagttctaaagagactgcaataggttttctaaaaataagggagggattaaccctcctttttataattttttgagttctggaaaaatccttaattagttcaagtttcgtaaagttctcttgatcttttccattctcttcttaacttggatagcttcttcttcgcaaggagcatggccccctaggaattggtgccatcttctttcaagttctctgtattcagattgaagttccatgaactcaagtgaatgattgtccatactatcacctcctcaacactattataagtgatactgtcatattctgtcaaataaaaaagagagaatgttattctccccatcttaatatctttatagttgctccatcaactcccttgccatccacatcatggacatacttatcaagtctcattgttgagtcctgtataattcttttgtcttctctgtcaaaaaccttaatgacatcagggttacccctgtcaatgatgtaagcaatctcttgagttccatctgcatatgttacttgaagtaatgaatgtagaggaataaagtctggagctgcccaatcaccaatcttaagatcccctcctatactattcttggtctcatatcctgccacatctgtaggctcatctgatgagtaataagtaacttcaactttgaactccattcctttaaatgaatttatcatctcaattagattttgtttatcagttctcagtttatcattctgatattttaatccttctacattgtccatcagtatttcagtctgctcagttaattgtttattcgactcaatatattcttggacagcatttccccaatgattgtttaggctctgtatggttaacagtagccctcctatcacaattattgttagtaatgacataattcttttaatcattctcttttaactcctttatttttaatttgaatttctcaattccagatttatacttacccacaatatcaaaggtatcggttagtattgcataggtttccccatcagaattaaatctgaagcttcctctcttgatgtctcctagcttattaaaggtcttaccctccttgtccagatatcctttatagtccatatagcacagacaagcagtaacaaactcctgcttattcctgaaattatgcttgatacccataccatctacccatttacttaatacaaatagactttcattagtcttctttactttactattctggattagatccttccacacataatcattagcctctttaaatgacttaaatctcttgcctttcagtatcttactactctggatcttggctttataatcctcaaatatacttggccagaagtcttttagatataaatacaaggaaatatcatctaatttagcattcggatcgttaatctggattacaggatgaccatccattgctctgatattattccttagttgggtattctctctcttcattttagatacttcaatatataatttaacgaatgcgtcagacaattcatgattggttaattccctttttaggggcttaccatctttactttctttagtagttacaatattaaagtagtcttgtaacctatcccagttattcttcattagatctacctcctatgcttacattatacatatattgtactgatatgtcaaagtccaggcattaactgatatctgatatgcctatatttttaccccatatcagtctgatatcccacatatcagttgaaactacaaaatcacaaaggcattggtatcactggcgtagagggatatcagttatgccccctttatatatacatagtattatatatactatataataatatattattatatatagtatatatatattacatggtgattacatcaatggcaggctattgccttgcctccattatcattacggcaggcatatccatgcttccgagcttttgccctatatagaaaaacccagacggtcagcgatcgagctcttgattttgttttgtcgagggagagaacagtaagagagaacccccgaacgttgacagttgtacttacttctcttataatgacagtaaaggagggataaccatgaaaacattatttactgatacaaaactagtattaattgaaactactaacttcttcattatgttacaagaagaaggtaagtatgtactatctaaaacaatcgataaggagatgggagaacaaatacacagagtatctaagttagctgcccttgtatatactaatgaggagtatactaactctaatgaaccaagatctatatacttagatgacaatttcttatacgaagtgcttggtaatgggaagtatattataagatacagtatataagagcccacaatcaattctaaggccttttagatatgtggtaatgtgattttacttataatgtggtagagacaccttacaggagctgctagaggcctttaaaggaggtatatcatgtatttatgtaatggtaaaatagtcaagaataaaaatgacttaaaagataagtttggtggtaaatcagtagtattcatcgatggggatgtagctacagtaatggactttagtgacagaaagccaaagataacaaaatatcttattagggaggtatcacatgataaacacatcattattgaagagactggaagggatagaggaaaagcataagcaaaatactgatgagataagaaagaacctaaactatgccagatatttgattgagaaacagtattgtcatttaacaaaagaacagaagataaaattgggacagttcttaggattgactgagaagaagttaaaagaaatacaagagataaataatcagttaataaatttgagagtggggctaagttatgaagtcgtatgtaataaccagaaaaaatagtggggtatctttagcagatacagacatgggacaagtattagctaagatactatgtaagcatgggggaacacttaccattgaggaaattgaaccagaacatattggtcaaactttttctattgtagaaggtaaaagaatatggtataatagaaaaggaggtgataatattggggagaagaagtgctatgttaattctcaagtatgactgcgaagaaactccagaaaggattgaattacgaaagaagtggttacagatttgtcttcattcaataatatattatagatatgacaacaatatctggacagaccaacaatgggatgagactgccagagaggtagttaaacttaagaatgagaatccaggtttagtaaacagtatgccatttaggaatgaccttaaagtctttgatggatccactggctttaacctttcatgtatgcaagatattaagatgttaaggtgggctcaaaacttacttgactttcatgttaaacgaggacttgatggaaagagtaagaaaaagaagaagaagaggaggaaaaagaaatgaacctacttgagcactatataaaaaaggtacacagtgtaagagagtaccatgaatttgataatgaaccttgggctaaaggtaaacaatatgtagaagtagacatggactatatttgttattctaatacaccacaaagagtgaagatggtatttactgttgatgagtgggagaagataaaatatagaggctactacatgggataggaggaatagttatgataagagaaatgggcatgagaatgctaataccagaaatacatgatataaaagatagggatatacaaaattttgtaagaaaggccctaaatgagatagttgatgaaaagttctttataatacctgcaagtagtactgggaaatatcatccaacttatagtgcaggggtaggaggtttgttaagacatactaaagctgcttgttatataggtaaagcattatgcgaagctgagatgatatgttcaagggacagagatatgataatagctgctttaatattacatgacattaataagccagataaagaacatccatatatggttagagagacactatcacccctagaggaagagtttccaataatatacaaagtggtagttgaactaattgagtctcatcatggtcaatggggtagtgttcctattaatagttattcccagagaatagtacacttggctgattatatcagttcacagaaaggtttaatattctcatatgaccaaggaactgattattctgacctgttatgggaggagaagtaaatggtgctaggggtaataaccctagtatcaatatttttactaggagtgtttataggttttgaggtgaagaaatggaactaggttttgcgatactagctataatagtatcaatatttttagaaactaaatatataaaggagtagattattatgtcaagagcaagagctgcaaggagaagagccgaaagagagaacaaaaatcttaatgttcttaaagctgtggacatcatgttagccttatcatgctatacattaaagaaggaaggttatggtaagactagaatgactaggtttgtggaagggatgagtaaacacacagaggagattgaaaagggaacacttaactatgaaaccataatgggagagattaaggatttagtaccaccaggtatatttgatttaggggaggagtcaaaggagtgatagtattgggatatttattatgggcatttagaatattaggcatacttgtaatagtatggtgtataatggaggcgatcagttgtgagcaataagttatattttaggtatagtgctatgaactctggaaagactactcagttaatccaggtagcacataactatgaagaaaggggaatgaagccattagtagttaagcccggaattgatactaaaggtggaccatgtataatcagtagaataggggtagcaagaaaggtggatgttcttctacctcctagagttaaattatcaaaaatactttctgactttgagtctaattattgggcagtagatgttatattaattgatgaggtacaattcttatccagagaacaggttgatgatctgttaaatttatcattacattatcctattatatgttatggattgagaactgactttaaaagggaaggatttgaaggaagtaccagattattacaagtggcccataatattgaagaattaaagaacatttgtcaatgtggtaaaaaagccacattctcaatattaaaataccagggtaaatatactgaccagggtaaccagatacaaattgataaccagcccgaaagtgttgaatatgaagccgtttgtaatgaatgttataataaattaattttttctaaataactcgttgacaggctatataggatatgatattatagtattgtaatcaaattacaaacaccaaccaaaactttataattagttaatttcaaactatactaaatttgttatttaaaaattaaaaatatggaggaatgattattatggcaaaaggaaaagcaaaatggttagaggaagcaaacaataaggagctaattgtaatcgtacaatctgctttaaattctggagatgagaaagaagttaaaaaggctttaaaagctattgtggaattagatgaaagaactcctgacacagatggacaaataactgtagaggaagcattagaatcattagaaatggctgtaggaactgtaaaggctgcataccaagcagaaatagatgctgtggaagatgaaggtgtagtagatgctgacttcgaagaagttgatgaagacgaagcagaagaagatgaaaatgatttagaatcattatctaaaaaggaattagctgctatggctaaagacttaggtatcaaaggagctaagaaaaaagataaagatgagttaatcgctttaatcaaagaagctcaaggtgaagaagaagacgaagaggaagaagaagaggatgaaactcctgactactctgaaatgactaagaaagacttaattgctcttgctaaagaaagaggaataaaagttaataagaaaatgaaaccagctgagataattgaattattagaagctgatgatgaagaataattctcatcaaataataaggggagcaaacttgctcctcaaattttttacttattttagaaacagatgttagagggggatgtataaatggcaagaggtggaaattcaacttatactaaagcagtatattgttacaacaataatagggagtatagatccttcagatatgcagctaaacagttaggagtatcggctgttagtataatgagagtagttaacgggactaaaccacatatagggggattagtattcgctgagatagaggaaggcactagaaaattaaagccaaggggagaagtagttccatacttgaaagaattaggttgggataatatagacttataatagggggtataatatatggacataaagttcttgaaggatatattctctaaacaatgtgaaaatggggattacattatcctagcagctagaaaaggtaaagaatggaaagatgtaccaatcaaatataataagaataacattgacaaaaaactaaaggactttgaacaacagtataagggttatgatttatattggagcccaatgccctatagtaatcctcaaagaaggatagttaacttcatagagactaaatacttaatacaagatatagatgagcatactgacccattggggattaaacctaaaccaagttatctgtgggaaagttctcctggaaaatatcaggggctatgggaaatggataggtatatagaggctaatcaatatgacgaaataaatccagcattagctaaacatataggctgtgactcctgctttgatgttactcatgtatatagaataccaggaactattaactataaatacaagaataaaccaaaagtaaaaagacctatacacactaaggagatatataagcctaaggtgatcgctaaggctgttaaggctgtaagtaaatctaatgatagtgttaaggtcaatataggaggatctgaggcctcacaatctgaaagaaagatatatgctaaatataatataccaaagaaggttagagacttactggctttagatgacattacttctttagatagaagttctactatatggtatattgagaataaattacatgaaataggactagagcctaatgagattatattattagttaagggctcagcttttaataaatataagggaagaaaagatgaagaaacaaggttaagaaaagaattggataaaatcataggaggagaaatagaggctgatattgaaaaggctgaaagtactaaactgagaatagatagttatcaggatgttatgggtaataatggtgccttcccaggttggttagtacaaggtttctggggtagaagatctcatggaattgtggctggacaaccaaaggtatttaaatccacatttacacaggacttagctatatcagttgctagtggaagacccttcctaggtcaatatcctgttctagaaccaggcccagtaattgtagttcaaaatgagaatgctgactggattatgagggatagaactgaaaagataattagccacagaggagtagttggtaatgtggatataaagggtaagagaagacttaaagttaggtttgctccagatcttcctatcacttttattaatcaacagggatttatgttagatgaagaatcccatagaaaacagatagaagaattaattgatgagataaaacctgtactagtaatattcgacccattatatcttatgtttagtggagatcttaataatgcagctgatcttaatcctgtactacaatggtgtcttaaacttaagaatgagaagcatacaggagttatgttaatacaccactataataaaggtggaaatgccactcaaaccagaggtggtcaaaagatggctggttcattcatattacatggttgggtagaatcagcattatatttaaaaagacctgatgacttagaaggtgacgatgaggagattgaagtagatatagataaccttgataaacaaagccatttaccaagtaaaatcattatggatagagagttccgtcttgcaggacaattccctcaaattgaattgaatttatcaatgggagaatttggagatccctattatcatgtagaagtagcaatacccggaaaagaagtaattgtgaaacctgaggacaaagccaaagttatagaggctgtaaaatcaggagctcataccaaggaggagatagtgtcaatatcaggattaaattcacagaaggttaatctagttctagatactttaaaagatactattgtatattctccggataaaggttataatataagtaagaaactaaatattgggaggaaaaaggcatgataataaagtgtaagaggccagcaggtcataatcatataagggcctttgtagtagtaattattgctagaggtaagaagaataaaatcacttatcattcaggattgaaatatttctatacctataaatcagctaaattatttatagacaaagttatggaagaatgtccctgggctgaattttattgggtggatgtccatgaagcccataagatccctgaaggcgaagagatacctaagaagaaaatgtggtgtccatattgtcaaactattcaagaatttaagagaagccaaggaggttacaagaattgccctatctgtggtataagtgaccaagacttttatgtaaaatgtatgaatataagatatagggaggctaaggctaatgcgaagaagaaacttgaaggaagtaatactaatcctagggatatcattgtcaatggggataatgctaactcagggggcaaaactaatagaaagtcatcaccaaagaaaaagtcaagaaaagttagtagaaaagcttcataatgctttagactataatgttattgagacttctccatctggactagatggggaggatcttattatcaaactaaaccttaatagtcctaaagaccttacccctaacaacttatctaagttagctaatgaggctatggtcaataacttaggagctcagaattatactatacttgtttatgatagtaatagaccagaaaatcttctggctgttatagatatacctaaaaattctaaaataacctttgacataataaattaattatggtaatataaaaatgtagaaggaggagaatttaatggtcaataaaaagtattacatcttgaaagaccttaatgatgacaaaccccaactatggaagggaagtttaaccactgctactaagatagcaggagcattaggagttagtgtgataaaactaaataggtatttagtaagaaagggatttgccagaaggtacaatgagcatacacttgagataatagacccaatccttgctaaagaacttggttattatgtaactccaagtaagtcccttataaatcctttatttgaatataatgataaaggagtacaatatatactaaacttaatagtagaagatctaaagaatggaggagagctttaatgattatcattttaggaatggataactcaggtaagaccacaacagctaagaacctaactaaacacagaggaggagaatatatccaatcaatgggacctggttcttatgaagaacaaagagaatgggtattaactcaaattgtgagaaaaggtgaaagggaagctatacatgatagatttacttgctttgaagaaatggtgtatggacctatcatcagagatagtagtaatttcaaccttgacagtaaggagctaaagatcttaaaacatctatgtaagccaactattgtatatgctagaccacctagggaagtgatcttcaattttggtgatagagaacagatgccaggagtaattgaaagagctgaacatctactggctagatatgatgaactgatatggaagttattctgtgatggatggaatgtactggtatatgattatactacttccaatgtggagaagctatcccagttaatagatgactcaagtgctaaagaagctataaaccaatttataaatatatcaagataagaggagagattgttatgaatataaaccatgcagtagaagaaaaaatagaaggagatagattacaagctatctttaatagacaaaaggagttaatggagaaatatcatcatatagaagctagatcaggattatgccaaactgaagactgtccagttaacttaaatgataaaagaggtcaagctagacttaaagattttgcttggagaatgactgaagaagtaggagaagcattggatgcttataatcatgaagaccattaccaagaagaattaattgatggattacacttcttaactgaatttacaattctagctggtaaggattataatactatagataataatgctatattagttgatagcctagagaacttatatcataaggctactacatcaccagaatttcctgaaatgttagtagaagaagctgtaactgacctggtaagagaaatgggtatgtgctgtaactgccttaagaataaaccttggaaacaaacttcaatgctaacagatgtaaatgcttttaatcaaagattattcaatgtatgggtatgttacattaaattattagctgtatctggcttagaggtagatgacatagtaaatatataccttaagaaatcacaggtaaataaattccgccaaagatctaattactaaaataaatacttaggagaaggtaatatgctaataagagactataatgattttgatgacttattcttaaaccttaatagggaaatgattaccaatccagaagaaactatgatgtatactcagaacatacagggctttcaggaggacttagttctctcctgtaagtcccataaatgtactttaaatctaggggactttggatataaagaaggtaagtggggacacctattaagatcatacattgattatccacaattaattgaatttagagaaaagcttaccaagataagtggtatgagctatacttattatttcaacaggaaaaaagctactaatggttcttgcttgatagctgcagtagtaactagaccaaaaagaaaaggaccttggaaacacttaaaaattatgtatagagtatgtgaattacaaaagaaattcgcagctgatctagtattaataaacaggttcattgaagaactacctcaagaagtatgtgagatagataatattacttttcatatgtctcaagcttatttgtcaggaatgtttataaatggatatttcaattattttaaggtaccaagaaagagtattgctaatagcaaacatccttggcataaatccttgaatagtaactataacaggttctttaaatcagaggaccagatacactcttataaagctctccagaagatgcagttactacattttggtctggagaaatttctaaagatagatatcaataaattatctattgacaagtactttaataagtagtataattaacttaacaaaattaaataaatggaggaattaaactatgagaatttatattaatgctcaagaagcatttgaagaagtaaaaagagatttatgtgaaatggggattgaggtaagacccaaaactatgcaagataaagttatagaaggtaatccagattatttcacaaaggagttacaaaactatagttacacaattctagaaagtaaacctgaagaagttccaggtgtatctcaaccttgggcagatgctgaatttagagaaaggatctacgatccacaaggtgtcatcaatcaatactctcttgaagaaagagaagaattatttggtatacatccacatcatactagggaggctttcataaatcccggtaaagcttatcaattaagacctgaggtatggaatgaatatctaagagatggaaaatttgggtattcttacaatgaaagaatttggcaatacagacaaattgaggatatcatcaatagaattaaagaagatccaggctcaagacaattatggttatctctgtggaatccagctattgatccattcaatataggaggagtaactagagtaccatgttcattaggatataacttccaagtaagagaaggtaagctaaatatccattatgttatgagaagttctgattttgctactcactttgctaatgatgtttatcttgctatgaaactattacattgggtagctgaacaaactggctatgaaccaggaagtttctctcatacaattttctctcttcatgtttacaacaaagatattaagggggtattctaataaatgagttacatgagaaaagaaagatataaacattctgatcttaataataaggttaacaagaaggaaaccctaaagcaatttattaggaatactgaaaaggaatttgatttagaaccagctaaccttggggacatgactaggaatgaacttaataactatataaattatatggatgaactgtggagtaagtaatatgtataattatagtgatgataacagacctaagaacaataacaatggctgtcttggttgtttaattataatcttagcagctataggattatgggtaataatttttgatattgccaatataatatatcatatgatattctaaatttaaagggggctatcctaatgaaaaatataatttgtcctatgtgtaaaaactcagtaacattaaaaagaaaatatggagctatgttttggatcatgattttcttaactggaggcctatgggtagtaaccatacccttcaaaaaacataaggtctgtccagtatgtaactcaatcataaaataaagataagggcctttaggggtcctttctatttaggaggtaatattttaaatgagatgtaacaactgtaacctatatactcactcagctccctcatgtatagaaggaacttgtgtaggaaagaaaaagaagccaagaataatggtcataaatagtttagctaatgatagggatgaggccaatagaatagctactcctgataaatcattacttgataaaatggaaggtctagacttttattataccaatgctattaagtgtagaactcctaagggtactaaaatcaaagtatcagagattaagaaatgccaagaacatttacttaaggaaattgaaaaatataaacccgaatatgttatgatcttaggatctcaagcattaaagatgctaagtaatgaaggtataacttcaatatgtggagtacctaagaagcatgagaaatatggctttaagtttattgccagctattcacccggtgtagttgcatatgacccaactaaagcacaatttgtagatcaggcctttaataactttaaagccatggtaaaaggtaaagagcatgaattacctgatcttaacataaaacttattactagtatgaaagaactaaaccaggctttcaaatatttaagggatgagggttataatagagtatcatatgatatagaaactagaggcttagataggtttaataataacattactctatttggttttggtaatacccaagtacagtatatactgcctttagaagtcaaatatagcccattaaggggtaagcccatagcacaaagaagattagctaaatccttgattaaaagacttaattctgagatgaaggaaagaatagcccagaatggtaagtttgatgataatttcttaaaggagaaatatggtattaagccaatcataacctttgatactttactagcctcacattgtttagatgagaatactcctaatggtcttaaggagaatgctttattacattgtaatgctaaagactgggatataaataagaaattaaagactggaaatgtggagactaaatcagactttgaggattatgttaggtatctggggtatgatatatactatacatttgctctatataaaatatttaataaaagacttaaaagggatgagagcttatataaactattccaccacttatacatcccagctagtaaagcttatgaggatgttcagttcaagggtatatatgtaaatcaggagaaattcaaagaggttgaaaaatacttaagatctgaactagataagattgagactggacttaagaagtatactaatggccaggatattaactggagctcacctaaacaggttggagaatttttatatgatacacttggtcttcctgtgattgaggttactgactctggagcaccagctactggagaaagtgtattattaagactaagagataaacatccagcagtagaactactattacagcataggggagttcatatacaaatttcccactttatagatggttggctaaataggatgcacaatcatagattatatccaaactttaaacttcatggaactgtaacaggaagaacctcaagtaataatcctaatctacagcaagttcctagagataagaaaatcaggagtttattaggaccatctcctggaagagtattcattgaagccgatctatcccaggccgaacttagaatagctgctatgatggccgatgaggataatatgaagtttatttaccagactggtggagatatacatgactccacatataatattatatctggggaagatatcaatgatgagaaagatccagcagttaagaaggagaaaaggaaaaaggctaaggctgtaaactttggtttcttatatggtatgcaatggaaaaaattcaaggattatggaagagacaactatggtcttaaattaacagatgaggaagccaaaacatatagaaggaacttctttaataaataccctaaactattaacatggcatgataaacaaagaaaaattgttaaagccaatggtgaagtaagatctctaataggaagaattagaagattacccgatatatattcatctgatagatctaaagctgctgaagccgaaagacaatgtattaactcaccagttcaaggttttggttcagatatcactttattaggcctatgtgagattacaggctatgctaaatatgttaatcctgaatatgtattagataagtctaagtttgatgtattaggctcagtacatgactcaatattatttgaagtagataaagactatgtggaagaattagcttggaaagtaaaatcaatagttgaaaataataaagtattaaagaaagtatttaaatttaccccaacagtcccaataatcatggatatatcagttggttattcttggggaggatgtgttgaactggattttaaaggtgattggaaaagccagataagaaaagtgttgacagatgaataattatctgataatataaatattgtaatgaaaaggaggtataaggatgttaaaaataagtaattccagaattaacaaattcttgtcttgtccttatgcccattatgttaaatactatgaaggtctggtacctaaaagaagtggagctgccttacaaaggggctctgctatccaccaggctatagaagactaccataatgggaagagttggaaaaaatctgttgataaattttccaaagagttttacaaaaatacatttaaagaagagatccttgaatttggagatattccaaaaatggtttattccttatgtgataactatttccactattatgatgaaaaagaagataatgtaacctatgtggaaaatgaacatcacttcgaattaaaactatgtaagggtgtaactctagaaggctatattgatagtgtcttagatgtggatggaaagatatgggctaaggaaactaaaacctacaaaaagatgcctgatagaaatttcctgatcttcaatagacaatctgctatatatacctgggctcttctacatgaatacccaaaagtaagtggtactatatgggatataatattagctcagcaaccaggtagaccagaattaactcaaaaaggggtattatctcaaaagaggattaaatccacacccctagagttagaaagaggaataagagaattaggattagatcctaaagattatgagtcttatattaattctgctagatgggaagacttctttgtaagacacccaataatattatcaaagaatatacttaacagtgtaatgattgatactattgagatagctaaacttattagagatgagggccacaaaagaaaggaaaagaaccttggaaaaggttgctctttctgtgaatataaatctttatgccaagctgaacttttaaatcttgataaagaatttattattaaggctgactacaaacaaagggaggaaagtgacaatggcaaaaaagcaaaaatcaaaatcaaatagttttgaggacagattagtggatctatatgatatagatgagcccacaatactaacactttatggaagatctggttcaggtaaaactactatctcaggaacactacccaaaccaatattctttattgatgtaaaggacaaaggtactctatcagctagaaacaagcttagagttaaaagaggagatatacaagtatttagtctaaagagttttgatgacatatacgaggcttatgattacctatcagaaaacactgataaatttaaaacagtagttatagaccatttaactgctttacaagaattaggtaatgaaaaggtcaaagctgaagaaggtaaggaccagatgagccaaagaatgtttggaaatgtggctaattatatgaaagaggttataaacctttataaagaattaaatgaggaaggtatactaccatgctttatagtacaagataggttagaatctggtgatggtgaaggagaagaccaattaatgcctgaggtaggaccaggattaatgccatctgtatctaaatatttatgtgctgtatcaagagtaataggtcatacttatttatatgaacactcagaaaaagagggtatgaaggttaagaaagaaatccagtatagactaagactaggacctaacccttattatattactaaatttactagacctcaaggatctgaatgtccagcttatctggtacatgatttaaaatcaccaacaactatctgggaggatattgaaactattctggctggtgaatggaataataagccagctaaatctggtaaaaaaaccagtaagaaatctggtaaaaagaaaaaataaaattttctaaaaatacctttgacaaccaattaaaaatctgataatataaacttgtaaacaaagaggtacaatatcttgacaaatatttatctcataatgatattttaaaatttaaggaggacaataacatggctaaaaagactactaagagaggtaacaaaaacaaaggaggattaaagattgatctttcaaacgttgaaacttcagttactatcccagaaggaaattacattgtggaagtagaagatgtagaggttaaggtttctgaaaatagtggaagcaattatttatcatttacttttgtaatagcagaaggaaagatgaaaggacaaaagttataccacatttgctcacttcaaccacaagctttatttaacttaaaaggtgtgttagttgctttaggatttgatatccctgatgaggagttcgaattagatacagaagctctagttggtttacaatgtggggtagaagtatcacatgaaatatatgagggtaagaagaaatcaagaataactgattttataaaccttgacgaagctgactctgatgatgacgaagatgaggatgatgactcagatgatgatgaagaagatgatgaagacgatgagtctgaagttgatcttgaagaattagacaaggatgagctaaaagaattagctaaggctttaaaaatcccagctaagaaaatcaagaaggctaaaactgaagaagatctaattgatctaattgaagaagaagctgacgaagaagaaatagctgaacaatataatgacctattcggagactctgatgaagatgacgaagaagatgaggatgaagaagaggaagatgaagaagaaaatgactatgagtcaatgactttaaaagaacttaaagctgaagctaaggacagaggcttaaaggttaaaaaaggaatgtctaaggatgacatcatagaaatgctagaagaagatgatgaagaataaaatttaattattaaaatatgagggcctttaaggtcctcctttatttacccttggaggctactattatgcttgaaagagatgtggttaaatccataatgaatatgcttaaaaaagaatacccaggtttttggtttaaaactcatgggggaccatttcaaatagctggcttacctgatatactaggttgccacaaaggtaagtttattggtattgaagttaaacttcctggaaaagaaaagaacctaactcaaaaacaaaaagacattataaataaaataaatctagcaggaggaatagcttttatggctacctcagctgaatatacaaggaggagattacatgaaaaatttagaaagacaccaacaattcctaggagaactaggagatctgtatgaattaaagaataatctatatggggataatttccacaagacttatcttgaatatggaaaccctgttctatgtataagacttgaagataagctaggaagagctaaaagtttattactaggagatcaagatgacttcccttcatatgctgctcaaaaagaatctgtggttgatactttactagacctagctaactatgccattatggctgctatggaactaactagtgatgataactcagaaatacatgatcttagtaaagaagaatatgatgaagaagacctagatgataatgacgatgatgacttagatgatgatgacaatgtttacgacgaagaagaattagattttgatagtatgaataaagaatccttaaaacaatatctaaaagataatggggttaaattccatagtaaggcctcaagagatgaacttgtaaaactggctaaggaggtataaggaggaggctttaatgcctcttcttttttagtatgaagagaaaattatttaaacatcagaaagaagcattacaactatttttaaataaagaaaagtttgccctatttatggacatgggtacgggtaagaccttagtccctattgtggcccttgagaaacttgaaggtctagatactgtactaatattctcacctaaatctattgtatttaactgggagtctgagatccataaatttactaaacttaaggaatataggatatttaaattacagggtaataagaccaaggttatggaaacctatagagctataaaatcctactcaggattaaagattattattgccaattttgagaaggctaggttgatggataaataccttatgaacttaaagccacagtttattgttgttgacgaatcccataaggtaaagaatagaaatgcccagatatctaaggctctatataaaattgctactaaatgtaaatataggttgataatgacagggactcccactcctaatggttatgaagatttatttatgcaatataaaattatgaactcaaatattctaggagttaattggaaacagtttgaagatgactttataatcaaaggaggttatatgaactatgaaattgtggggtataagaatgaggaaatattaaagaaccttatgcaccagaattgctatatagtaagaatagaagattgtattgatttaccagaacaacttcctgatctgtatttaacctgtgaattaaatagtaaagccagaaaggcctataatgaccttagaaaggaaatgatagcacaactagatatagtacaggaaaacattcctagaaagcaattaaaggccttattaaggtctaatggtataccctatgagagtaatgagccctatgaggatttattcttaagggctaatatgtttatcaaccaattaacagctgatcttactattacccaatatttgaggctacagcagatctcaggaggatttatcacaaacaatgtaggaaataatattaatattgataaaggcaaattaggcttgttacaggactatctagaaggatataaaaagcctgttgttgtaatatgtaattttcttgaggaaataaaacttatacatgatacttttaaaaagacccacagagtagaatgcttaacaggatctactaagaatagagctgagatcaataaggattttcaggagggcaagattgatatattaatactacaaataagctcaggtagtgttggtctaaacctcttcagggcctcaaggttaatattctatagttggaactataaatatgatgattatgtgcaagctattgccagaatcaaaaggaatggtcaaaaggagccttggcaaataatacacttaataacggagaatactattgatgagaaaatattaaaatcaatacagcttaaaagggatagagcagaaaaactgttgactattgataagtaatgtggtaatatagaattgaggtgataagtaatgagaaaagaacaacctagaataagtaatcatactgaaatagctaaggctttaattgaggctggtaaaactattaaagctctaaccaagattaaagtcaaggaggaaaagaaaaaacaaaaaagacttgaaaggttaagactcctaaatgaggaaaagaagaaggagagagaattaatgaaagaatttaatcccgatgagcctaagaagccaagaaagaaaaaggacaaacctataaagaaggttgatctgaataaagttgaggctaagggaacttaccctacaccttctggaggtaatgcacctacgggaacagttgacttaaaaattttatgtgagtcattaggattagatccaagtaaagccagggccaagctaagaaagcaaggtgtaaacaaaccctataaatggtcaggatctgaacttgaggatattaagaaaatgttaaaataagggggaggtttaaaaacctcttctttttcgttgacaatatccacagtatatggtaatataaatattgtaatcaaacaaaaaaaggagagaactgaatatgaaagatcttgaaaaacttacaagggaagaattgattgaacttgtaaaggagttatctattgattggacaggagcctataatagaaactataagattgaccttgatgagtatgagattgtatatattgatcttaatgatctaaaagagttcaatgataaattaggtcatctagaaggagatgtgtatatacaatacacggtaaatcttattaaggcccatttacatcctgagaaggatatattgattagagggggtggtgatgagtttgtagttatcagtgatatagcttataatctgtgcaataccttgaatatataccctgagctatcatgtggctatggtaaaggtaaaactattgaagaagctatagtacaggccgactcaatgatgtataagaataaaaaatctaagaagttaagatactcaaaggaggattagttattatgaggttattatggttaaaagaatatttggatatatgcaatatcttgggtattgagcccacaatggaatcttgtgctaggtggggaaagaataaaaaactatcagggttttcattaaccccagtgggagcaactaaatagttgcttctttttaaagcgatccgatacctagcaactttcatgccaaaaagaaattcgggattttctttgacatagactccagagtctggtataataatcttgtaaacaaaattaattcaaaggagttgttaattatgaataacaaaaaatttcaagaaactttagaacaattaaaggaggaactagaaatacaaggggtagaatttaatgatgagaatgacttaatagctgctgttgaatacatcatagaatatgattaccacccagaacaatatgtggaagatactttatgtaactaccctgaaatgttcaaggatctataaaactaaggaggtgtaaaaacctccttttttatttttctaaaaatctggatttaatcgttgacaggatcgggactatctagtataataatattgtaatcaaaattaattgaaggagatgttaactatggaactaacaagatcagaaaaacttaatgtaataaaaggaattgctcaaaaggctatggataataaaatctatccacaatttagaaaagaactagataaacaggtaaaatcctttggactaagcaacaaagttagggaaagtgaattaggagactacctttcttgctgtatggttgcctatgaagaggttatactaaaaatgaaaaaagccaattaatatgggtggccaaaaggccatctatttttttcgaaaaaatctccagaatctcgttgacatagtctgggccctctggtataataatattgtaatcaatattaattaattcttaggaggaatgaaaaatgactaaattagaaatgttaaatgagatagaaaaaataaataaggtggtttttgaaaagaacttccaaaaacaattcttggataaggtgatagaactactacaacaaatgggagtaactaaatattatgtatgtaaacatcataaaaaagctgagattgaaaaacatcttgaggcttgcatctgtgcaatatatgatataggaagaagggatgatctaggatggtaaaccccatcctttttcttcgaagtttttcattgacagatccagagttctctcttataattaaatcataaattaactattggaggtaaacaaaatgagagatatgatagaaaatcaattagctgaatatgaggtaaaggagttatacaatgaggccacaatgatcttaggaaaagcatttggtgtaagtgctgttgatctttatatagaatctgatgtggatgctaactactatggtctatgccatagatcaggtaataaatttactgggattacaattaaccttttccctttcaggtttgcacaggaaggagaaaaagcttatgataaaatcaaaaaatttggctgggatattaaggactgtgttcttgaaactatatgccatgaattggctcacttaacttattggtcacatagtcctttacataaaaaattaactagtctttattacaacaaagtgcaacaggctagaaaaggtgaaaactcagctgtagcacaaactagaagtgatatatacactttaaaagatttatgtgaattaatagaactagatccaagaaaggctagaagtatattaagaaagaataatattgagaaacctggtaaacagtgggagtgggagcaaggtatgcctaaagatatatatgatctattaatcaacttaaaggttaggggaagaaggtaaacttcttctcttttttcgttgacatatctcgagagtgctggtataattatattaacaaataacttagggggtaaatcacatgatagatatatattatagtattcaagtagaagctgaaaacttctttggttgtcaaaaagaagatggaagctgggtagcaacaggagcatttagtatacctgttaatagcataacttttgaagaggctgatcaattatccaatgaggccatagatgggtggttaaaggagtatgaggttactaaggtaataagtaggagatcacatacacaggttaaattagattggtataatagttatatcaaggatgatccattaaagggtgatataattaatatggtgtaccctgatctttcagataaagctaaaatcaaatatggctttggtaagataggggctagcactatgtcaaaggttgctaagaagggtttacttaaaacttgccctagatgtggaggcactggccattgctcaagaacctcagatggtaacactacttgctttaaatgtaagggctttaaatatgtgataccaactaagatctcaaagaaattttataaatctgtggagaaaacctttgacatctctggcaataactcttataataaacttgtaaacaaaaacaaagaggagatgttaaatatgaacttaactgcaatggaaacaaagatattaaatgctatgagaaagaatgaatttgatgatggactagatgttgactgtgtatgggtattctcagtaatagaaaactcaggtatagaaggaactaaggctagaggtgtgatctcatcacttgttaaaaaaggtttagtatttgctgatggagaggtaataggttacacagaagaaggaagaaaggtctttgataatgctgatggagaagaatgtaactggggaggtccaaaattattaaaagaaatccctgacaaaccagaggaaatctcttataatgaaaatgtagataaaacaaataagaaagaagaggtaaatgatatgaaagatttaaatactatgaaagctgttgaaattaaagaattagcaaaggaattaaaagttaaaaactggtggactatgaaaaaggctgatctaatagctgctatccaacaaatccaacaaccacaagaagaaaaagttgaagaggtacaacaaccagctgaacctgaagaaaaggctgaacaaactaaaattactcttgatctaacagatgttaaggaacctgaagaagaaaaggttgaaactaagaaaaaaccaaaaactaaagaaggtgtatttacactaaagatgatacttgaagaattaaatatgaatggtaaaaaggcaagaaggatcttaagaaacaaagaggttgtaaaaccaggaaagcaatgggaatgggataatgaagaagaatttaaaaaggttaaggacctactttctaaataaagtaggcccaacctctatcccctattgatttacaggaggatctgattttctcttatccattaactgcttccatacttgattaccaaaggaagctacagctgcacatattaaaccctgtataaagccattcaaaaaggtcttggctgtaaaacctaattctaattgaattgccatatataagattgataatgatatactgaatatcaaaagtattaatggtatagaccaatctggtatataaggcttagccttgataaacagacctaaacagtaacatgatacaatgattattaaaagctgtggatcaatgtaattgaatattaagtttactaaattttcttccatgataaataccccctaaattatctctacatattttgaacttacataaccttgcttcttaccgtggctagtattatattctatatgataccaaccattcttacttcccaatatagtaactctctcattactaaatactgagcctattatattaccattcacatcatctcttacattaagagaagtgttaactttaactattccttgtttaacatcctcatagaatttctggctttgctcaccctcgtagcgaacgtatccatcagatggagtaccatcctttctataaaatgttattcttaaccagccattagttctatacattgggctagccttttgaccaggctgtagttcttcattatgatctttgatgttaacgtcttcagggttccaccacacataagttactccattgtcattttgatatttcatgtggtagtcaaaacttaatctgctgtaatgttttatgtcaatataagcatggtacttcttattctttccaggatatacaacttctatgaaatttctagaaggatatattccgagaacaaataaattatctaggctatcaataaatctaccagggactggcttacaatcctcatctagaacttctattgaaccttcccccactaaagtagcattagttcttgtctcattagactcatagaatcctttggggttattgattactggtgagcttgagctctctcctgaatttactctttctaggaatgtattccagtaaccattggctatcattcttctaggacaattttttctactggcatcatagtgtcttactactttacaattagaatagtagccattctttaggtatctaactagctctacagcattatcaactgccttattgtagtcagagtcaggattaacacatatttctatagatattgtatttctattattgataccgtatctattatgaccatctccacaattccaagtggcgtgtttgtgttctacagcttgatatacccctgtatcatcgacataataatggacactggctttacctatatttccatttgcttgagccttacagtgggtttcggctccagcaccccaagaggtattatcagtttcgtggataattatatacccaggattatttgcatttagagtaacattcgtagtacttaatcttttattgattttcataataaacatctcctttatatattatagtgttttattgggcctgagaggctcgctacagcattttaaccacctccttaatatatttccttatataaaacctaacaggccttaaatggcctgctaggcttataagttaacctttgttactaaataggtgatcttttatagtatctacatcctctttgatatcctcaactacattgaatttatcaactagcttatctatcacttgatttaatttattctccctttctctagcttcttgtctagtgtcatataatagccatacaaatagactacaaaagataccttggctaagaacttgagttagtatttctttttccatagattacaccctttccttaaagtcttcaccacatattcttttatagtcctctggtgtaatttctccttccggattagaagagcattttaccgcctgatgtaatttgtccttacctattgctccaattctataagccatttcccagaaattcataatccctacctccttatttattcatcattttaatctttatatcagctagttcttgtgttaatactttcattatggccttagtttgcattagctctaatttagtatcagcaagagcctgggcttgataaccaattaatttattaatatccagaggattaggatctatagcctcataggaagtaaataggtccttatctttgatactgtatagatctgatctctttttactaatatcaaatttggttgggccaccctttatgtggtcaaataaacttacagtcatttgtatggctgaaagattgtctagatcaattacctcagtgttatccacaaaggctaaatgcccttgtgaattatgaggtatatggagacatataatatcttctatattatttaatatttcactatcctctctatagtatagaggttcaggcctattaattaggtctaatatcttagtaacttcttcatggtctttatctataaatgattttacatcttctgagtcttctgcctgatttatcagcatttctttttcatcatcatagaatataaggtctatgattttattagtttccacagaataattaaatcctactattctcatgttttatcaactcctttactcagtggctaaataggttagtattatttgagttggcttaccagctaccatttgataacatccaccattcaaatatgagttattccaatagtcaatagtacaataacctgaggtattattagaagcgtcattatagttatgtgatactagagatataggtaatacccaattccaagccttaggaaaatgtatagtataacttacacctccacctgagttagcataacccgtcttaactatttgacggactaatcttagtcctcccccaagatgacatactctaacgttaccattgtcattatcccaataatctcctttagcaatagatctattatttacaacgaagtcagtaacattctcagtatatagctttttgttctcttgtttgaaatacaatcttccatcttcagctccaccataccagtcatttattcttaggtattttctagcccataggttttcagctgatagagccttatcaacctctagagatccgtctctagtagttatcctcatatcaaaatctttcttactaccctttaagtggaaatctaatataggacctagttccataactccatcatgtgatataaaagggatacctgcatagtcattactagctccagctaagtcccattcttttagtttattactgttagcagctgtagcggttttacctaaataagcactatcatggttatggtctgaggctgcagctcctatatcggatggcttaggtttattgaggttactataagctatacaccattcggaccatatgcctttaaaactacaaaacctagtatatgttttgccataactatctgtaaatagttgagttacctcaccccccttgggtaataccaatagagttccataaataccatatgtgtaaactacaggggagtttggtaaggtatctacactagatactgagtatatcccctcttccttacaaagattaaaatctactatatcatcttttctaatagttaaataaactccctcatgggtatggttagttggggatgcccccacatctgctgcagttggtttattatcttcatgatagaccttcttattgttcttattaacaatatccagagagtctatctttacaggccttccagcataccctatatggactttattatctgcatctatatagatcacatagtcatcactgccttctttagtcctacagctaaatccataattgtgggccccaataaatttctgacccggtctcatgattagatggcctgataattctccacccgtagtaggtaaggcaccaatatctgctggagtaggcttattttgtttactatatatttcagcccaattcgtccatccggtaccctcaatgtttgtagctgttctagtaaaaactcttccaccatctgcaaagaacatttgagaagcccagtgtcctgtattccaggataaaacaatcaatctcccatctgctaggattggggcatttctatcgacagaatttctaactgtagaataaatacctccctctgtaatggtgtttagatctacaccctctagtcttttggctgttttatcccaggccccaatatctgcgggtgttggcttagctccggagttataatcttttctccaagggaaccaatccgtattatttactttatacctccaatacttattaccattagtatcataatactcttgccatatccagttattagtattattatgcttagtctctgtactaacatatactatcagtataccatattttgtaccagttagtggggcattaggtaactcacctgagatcaggtattgcccctcagttaaagctgtattaaaatcagttatggcgtccttaggaatgggataagcctttaggtcagcaggggtaggcttattagcctcatcataaaccttataccacttactccaagaattatttcctgatgtgtagtttctaacatatctagttattttattggttgggtataggttaataaactcctgttggaatcccctctcacctgtatttctaaccataaaaaccctattactcatatgggctaaggttccctcgggggtatttttaaagtcaccagttcctgtatcaaagtagaagaaggcattcgcttgtttaaaggaattacaatctctatctaagggagcactaaccttaataagtgcttgatcttgattagcctttcggtctacttgattttgtaaactggtgtctttctcaaataataggtctaatctttttagcacatcctcaggggctagattataatcaggtactacattacccctagctaatatgaggtttagtacctttaatgaggtacttgaggttgcactctgtaccacaaattgtattttggtatcagtagctccagatggaatactaaatttatgagtttttaacttgtacccattactctgtggtgtactaccttgttttacaatactcctatattgttgacctccattagtgtaagccagtttaatttcatagctagtaaaactaccttcaatatcttctagaaaggctagtatataatcactatttggttctataggcagagttttaatctcaagagtttgtggacctgttgacataccagaccatttaaaacctcgtctctgggttggagtatctgtaatgggtgtgatattaccaggaccagtataagactcagagttgtaccactcaagcctattaatagtaccaacccttaaagcatctagcctatcctcattagacttagacttcttttctacctcagtcattttctgtttatgttcggtagcaaagttctcaatgttctcattgtccttgttaaaatcattcatttttggcttatctgttaactcccacttatttaaacctagggtaggagttttactagtacttggcattttgcatacctcctttattcagttatagcatattcttcccatttttcccaggtaagatctagactgtcccacttgctccacatataatcatatctatcgaacatctcccaagtaatataaagtaatataatttgatatattaggtgagcaggcattcttcccctgaatactctttctagagcctttaggttaggtggtacccctggtaggtcagtaaagctaatcttgatcttactctcttcagctatgaactctacctttacctttccacctgtataggccttagtaagatttttgatagatgtactattaaactttttccaagcagatagaactactgtaataatagctcttttctcttggtcagttggtgggtaatcaaagtatttatataactcaagatcagtaaaaaatctttctagaccttccttaggagtggtcttgggatccacatagtcttgtaattcctgtcccttagtat